European Patent Specification EP 3 664 833 B1, published May 31, 2023. Title: GLP1/glucagon receptor agonists in the treatment of fatty liver disease and steatohepatitis. Applicant: SANOFI. The sequence listing filed with the application follows.

SEQUENCE LISTING (4 sequences)

SEQ ID NO: 1 - protein, 39 aa, Artificial Sequence
  Exendin-4 analogue
  MOD_RES (2)..(2): Xaa is D-Ser
  MOD_RES (14)..(14): Lys is functionalized at the amino side chain group as Lys((S)-4-carboxy-4-hexadecanoylamino-butyryl)
  MOD_RES (39)..(39): amidated C-terminus
HXQGTFTSDLSKQKESKAAQDFIEWLKAGGPSSGAPPPS

SEQ ID NO: 2 - protein, 39 aa, Artificial Sequence
  Exendin-4 analogue
  MOD_RES (2)..(2): Xaa is D-Ser
  MOD_RES (14)..(14): Lys is functionalized at the amino side chain group as Lys((S)-4-carboxy-4-hexadecanoylamino-butyryl)
  MOD_RES (39)..(39): amidated C-terminus
HXQGTFTSDLSKQKDSRRAQDFIEWLKNGGPSSGAPPPS

SEQ ID NO: 3 - protein, 39 aa, Artificial Sequence
  Exendin-4 analogue
  MOD_RES (2)..(2): Xaa is D-Ser
  MOD_RES (14)..(14): Lys is functionalized at the amino side chain group as Lys((S)-4-carboxy-4-octadecanoylamino-butyryl)
  MOD_RES (39)..(39): amidated C-terminus
HXQGTFTSDLSKQKDEQLAKDFIEWLKAGGPSSGAPPPS

SEQ ID NO: 4 - protein, 31 aa, Artificial Sequence
  Liraglutide
  MOD_RES (20)..(20): Lys is functionalized at the amino side chain group as Lys((S)-4-carboxy-4-hexadecanoylamino-butyryl)
HAEGTFTSDVSSYLEGQAAKEFIAWLVRGRG